European Patent Application EP 4 681 780 A1, published January 21, 2026. Title: IMMUNOCYTOKINE FOR CANCER TREATMENT. Applicant: EGLE THERAPEUTICS. Application EP. The sequence listing filed with the application follows.

SEQUENCE LISTING (41 sequences)

SEQ ID NO: 1 - protein, 133 aa, Homo sapiens [sequence omitted]

SEQ ID NO: 2 - protein, 124 aa, synthetic construct
EVQLVETGGGLVQPKGSLKLSCAASGFTFNTNAMNWVRQAPGKGLEWVARIRTKSNNYATYYADSVKDRFTISRDDSRRMLYLQMNNMKTEDTAMFYCVRGGYGISAHNTMDYWGQGTSVTVSA

SEQ ID NO: 3 - protein, 8 aa, synthetic construct
GFTFNTNA

SEQ ID NO: 4 - protein, 10 aa, synthetic construct
IRTKSNNYAT

SEQ ID NO: 5 - protein, 16 aa, synthetic construct
VRGGYGISAHNTMDYW

SEQ ID NO: 6 - protein, 112 aa, synthetic construct
DIVMTQSAPSVPVTPGESVSISCRSSKSLLHSNGNTYLYWFLQRPGQSPQLLIYRMSNLASGVPDRFSGSGSGTAFTLRISRVEAEDVGVYYCMQHLEYPFTFGSGTKLEIK

SEQ ID NO: 7 - protein, 11 aa, synthetic construct
KSLLHSNGNTY

SEQ ID NO: 8 - skipped

SEQ ID NO: 9 - protein, 9 aa, synthetic construct
MQHLEYPFT

SEQ ID NO: 10 - protein, 124 aa, synthetic construct
EVQLVESGGGLVKPGGSLRLSCAASGFTFNTNAMNWVRQAPGKGLEWVARIRTKSNQYATYYADSVKDRFTISRDDSRRSLYLQMNSLRAEDTAVYYCVRGGYGISAHQTMDYWGQGTLVTVSS

SEQ ID NO: 11 - protein, 10 aa, synthetic construct
IRTKSNQYAT

SEQ ID NO: 12 - protein, 16 aa, synthetic construct
VRGGYGISAHQTMDYW

SEQ ID NO: 13 - protein, 112 aa, synthetic construct
DIVMTQSPLSLPVTPGEPASISCRSSKSLLHSNAQTYLYWFLQKPGQSPQLLIYRLSNLASGVPDRFSGSGSGTDFTLKISRVEAEDVGVYYCFQHLEYPFTFGGGTKLEIK

SEQ ID NO: 14 - protein, 11 aa, synthetic construct
KSLLHSNAQTY

SEQ ID NO: 15 - skipped

SEQ ID NO: 16 - protein, 9 aa, synthetic construct
FQHLEYPFT

SEQ ID NO: 17 - protein, 124 aa, synthetic construct
QVQLKESGPGLVQPSQSLSITCTVSGFSLSSYGVHWVRQSPGKGLEWLGVIWSGGSTDYNAAFISRLSISKDNSKSQVFFKMNSLQADDTAIYNCARNKVFNYYGSRYEVMDYWGQGTSVTVSS

SEQ ID NO: 18 - protein, 8 aa, synthetic construct
GFSLSSYG

SEQ ID NO: 19 - protein, 8 aa, synthetic construct
IWSGGSTD

SEQ ID NO: 20 - protein, 20 aa, synthetic construct
CARNKVFNYYGSRYEVMDYW

SEQ ID NO: 21 - protein, 107 aa, synthetic construct
EILLTQSPAIIAASPGEKVTITCSASSSVVYMNWYQQKPGSSPKIWIYGISNLASGVPTRFSGSGSGTSFSFTINSMEAEDVATYYCQQRTSSPPWTFGGGTKLEIK

SEQ ID NO: 22 - protein, 5 aa, synthetic construct
SSVVY

SEQ ID NO: 23 - skipped

SEQ ID NO: 24 - protein, 10 aa, synthetic construct
QQRTSSPPWT

SEQ ID NO: 25 - protein, 124 aa, synthetic construct
QVQLVESGGGVVQPGRSLRLSCAVSGFSLSSYGVHWVRQAPGKGLEWLGVIYSGGSTDYNAASISRFTISKDNSKSTLYLQMNSLRAEDTAVYNCARNKVFQYYGSRYEVMDYWGQGTLVTVSS

SEQ ID NO: 26 - protein, 8 aa, synthetic construct
IYSGGSTD

SEQ ID NO: 27 - protein, 20 aa, synthetic construct
CARNKVFQYYGSRYEVMDYW

SEQ ID NO: 28 - protein, 107 aa, synthetic construct
DIQLTQSPSSLSASVGDRVTITCSASSSVVYMNWYQQKPGKAPKIWIYGISNLASGVPSRFSGSGSGTDFTLTISSLQPEDFATYYCQQRTSSPPWTFGQGTKVEIK

SEQ ID NO: 29 - protein, 124 aa, synthetic construct
EVQLVETGGRLVQPKGSLKLSCAASGFTFNTNAMNWVRLAPGRGLEWVARIRSKSNFYATHYADSVKDRFTVSRDDAQRMIYLQMNNLKTEDTAIYYCVRGKETGQNFYAMDYWGQGTSVTVSS

SEQ ID NO: 30 - protein, 10 aa, synthetic construct
IRSKSNFYAT

SEQ ID NO: 31 - protein, 17 aa, synthetic construct
CVRGKETGQNFYAMDYW

SEQ ID NO: 32 - protein, 112 aa, synthetic construct
DVVMTQAAPSVLVTPGESVSISCRSSKSLLHSNGNTYLYWFLQRPGQSPQLLIYRMSNLASGVPDRFSGSGSGTVFTLRISRVEAEDVGVYYCMQHLEYPFTFGAGTKLEVK

SEQ ID NO: 33 - protein, 124 aa, synthetic construct
EVQLVESGGGLVQPGGSLKLSCAASGFTFNTNAMNWVRLASGKGLEWVARIRSKSNFYATHYADSVKDRFTISRDDSQRTLYLQMNSLKTEDTAVYYCVRGKETGQQFYAMDYWGQGTLVTVSS

SEQ ID NO: 34 - protein, 17 aa, synthetic construct
CVRGKETGQQFYAMDYW

SEQ ID NO: 35 - protein, 112 aa, synthetic construct
DIVMTQSPLSLPVTPGEPASISCRSSKSLLHSQGQTYLYWFLQKPGQSPQLLIYRLSNLASGVPDRFSGSGSGTDFTLKISRVEAEDVGVYYCFQHLEYPFTFGGGTKVEIK

SEQ ID NO: 36 - protein, 11 aa, synthetic construct
KSLLHSQGQTY

SEQ ID NO: 37 - protein, 9 aa, synthetic construct
FQHLEYPFT

SEQ ID NO: 38 - protein, 132 aa, synthetic construct
APTSSTKETQEQLERLLRDLQLILKGINNPKNPKLTRMLTFKFYMPKKATELKHLQCLEEELKPLEEVLNLAQSKNFHLRPRDLINNINKIVLKLKGSETTFMCEYADETATIVEFLKRWIAFCQKIISTLT

SEQ ID NO: 39 - protein, 132 aa, synthetic construct
APTSSTKETQEQLERLLRDLQLILKGINNYKNPKLTRMLTFKFYMPKQATSLKHLQCLEEELKPLEEVLNLAQSKNFHLEPRNLINNINKIVLKLKGSETTFMCEYADETATIVEFLKRWIAFCQSIISRST

SEQ ID NO: 40 - protein, 132 aa, synthetic construct
APTSSTKETQEQLERLLRDLQLILKGINNYKNPKLTRMLTFKFYMPKKATELKHLQCLEEELKPLEEVLNLAQSKNFHLRPRDLINNINKIVLKLKGSETTFMCEYADETATIVEFLKRWIAFCQKIISTLT

SEQ ID NO: 41 - protein, 15 aa, synthetic construct
GGGGSGGGGSGGGGS